European Patent Application EP 4 786 491 A2, published August 5, 2026. Title: TL1A-Binding Molecules, IL-23p19-Binding Molecules, and Bispecific Antigen-Binding Molecules, and Uses Thereof. Applicant: NEWSOARA BIOPHARMACEUTICAL TECHNOLOGY (SUZHOU) CO., LTD. The sequence listing filed with the application follows.

SEQUENCE LISTING (119 sequences)

SEQ ID NO: 1 - protein, 10 aa, synthetic construct
GFTFDDYAMH

SEQ ID NO: 2 - protein, 10 aa, synthetic construct
GISWNSGSIG

SEQ ID NO: 3 - protein, 10 aa, synthetic construct
DSGAYVSFDY

SEQ ID NO: 4 - protein, 11 aa, synthetic construct
RASQSISSYLN

SEQ ID NO: 5 - protein, 7 aa, synthetic construct
AASSLQS

SEQ ID NO: 6 - protein, 10 aa, synthetic construct
QESYSYPPFT

SEQ ID NO: 7 - protein, 119 aa, synthetic construct
EVQLVESGGGLVQPGRSLRLSCAASGFTFDDYAMHWVRQAPGKGLEWVSGISWNSGSIGYADSVKGRFTISRDNAKNSLYLQMNSLRAEDTAVYYCARDSGAYVSFDYWGQGTLVTVSS

SEQ ID NO: 8 - protein, 108 aa, synthetic construct
DIQMTQSPSSLSASVGDRVTITCRASQSISSYLNWYQQKPGKAPKLLIYAASSLQSGVPSRFSGSGSGTDFTLTISSLQPEDFATYYCQESYSYPPFTFGGGTKVEIK

SEQ ID NO: 9 - protein, 10 aa, synthetic construct
GFTFSSYAMS

SEQ ID NO: 10 - protein, 10 aa, synthetic construct
AISGSGGSTY

SEQ ID NO: 11 - protein, 10 aa, synthetic construct
LEWLYGAFDI

SEQ ID NO: 12 - protein, 11 aa, synthetic construct
RASQGISSWLA

SEQ ID NO: 13 - protein, 10 aa, synthetic construct
QQADSFPPLT

SEQ ID NO: 14 - protein, 119 aa, synthetic construct
EVQLLESGGGLVQPGGSLRLSCAASGFTFSSYAMSWVRQAPGKGLEWVSAISGSGGSTYYADSVKGRFTISRDNSKNTLYLQMNSLRAEDTAVYYCARLEWLYGAFDIWGQGTLVTVSS

SEQ ID NO: 15 - protein, 108 aa, synthetic construct
DIQMTQSPSSVSASVGDRVTITCRASQGISSWLAWYQQKPGKAPKLLIYAASSLQSGVPSRFSGSGSGTDFTLTISSLQPEDFATYYCQQADSFPPLTFGGGTKVEIK

SEQ ID NO: 16 - protein, 10 aa, synthetic construct
SYEDTAHFDY

SEQ ID NO: 17 - protein, 11 aa, synthetic construct
RASQSISSWLA

SEQ ID NO: 18 - protein, 7 aa, synthetic construct
DASSLES

SEQ ID NO: 19 - protein, 9 aa, synthetic construct
QQYNSFPPT

SEQ ID NO: 20 - protein, 119 aa, synthetic construct
EVQLVESGGGLVQPGRSLRLSCAASGFTFDDYAMHWVRQAPGKGLEWVSGISWNSGSIGYADSVKGRFTISRDNAKNSLYLQMNSLRAEDTAVYYCARSYEDTAHFDYWGQGTLVTVSS

SEQ ID NO: 21 - protein, 107 aa, synthetic construct
DIQMTQSPSTLSASVGDRVTITCRASQSISSWLAWYQQKPGKAPKLLIYDASSLESGVPSRFSGSGSGTEFTLTISSLQPDDFATYYCQQYNSFPPTFGGGTKVEIK

SEQ ID NO: 22 - protein, 11 aa, synthetic construct
GQVAPLDHFDY

SEQ ID NO: 23 - protein, 9 aa, synthetic construct
EQYNSYPLT

SEQ ID NO: 24 - protein, 120 aa, synthetic construct
EVQLVESGGGLVQPGRSLRLSCAASGFTFDDYAMHWVRQAPGKGLEWVSGISWNSGSIGYADSVKGRFTISRDNAKNSLYLQMNSLRAEDTAVYYCAKGQVAPLDHFDYWGQGTLVTVSS

SEQ ID NO: 25 - protein, 107 aa, synthetic construct
DIQMTQSPSTLSASVGDRVTITCRASQSISSWLAWYQQKPGKAPKLLIYDASSLESGVPSRFSGSGSGTEFTLTISSLQPDDFATYYCEQYNSYPLTFGGGTKVEIK

SEQ ID NO: 26 - protein, 10 aa, synthetic construct
GFTFSSYAMH

SEQ ID NO: 27 - protein, 10 aa, synthetic construct
VISYDGSNKY

SEQ ID NO: 28 - protein, 11 aa, synthetic construct
GQVAILDYFDY

SEQ ID NO: 29 - protein, 9 aa, synthetic construct
QQYNSYPPT

SEQ ID NO: 30 - protein, 120 aa, synthetic construct
QVQLVESGGGVVQPGRSLRLSCAASGFTFSSYAMHWVRQAPGKGLEWVAVISYDGSNKYYADSVKGRFTISRDNSKNTLYLQMNSLRAEDTAVYYCARGQVAILDYFDYWGQGTLVTVSS

SEQ ID NO: 31 - protein, 107 aa, synthetic construct
DIQMTQSPSTLSASVGDRVTITCRASQSISSWLAWYQQKPGKAPKLLIYDASSLESGVPSRFSGSGSGTEFTLTISSLQPDDFATYYCQQYNSYPPTFGGGTKVEIK

SEQ ID NO: 32 - protein, 11 aa, synthetic construct
LGDGVTYAFDI

SEQ ID NO: 33 - protein, 10 aa, synthetic construct
QQSLDFPPIT

SEQ ID NO: 34 - protein, 120 aa, synthetic construct
EVQLLESGGGLVQPGGSLRLSCAASGFTFSSYAMSWVRQAPGKGLEWVSAISGSGGSTYYADSVKGRFTISRDNSKNTLYLQMNSLRAEDTAVYYCARLGDGVTYAFDIWGQGTLVTVSS

SEQ ID NO: 35 - protein, 108 aa, synthetic construct
DIQMTQSPSSLSASVGDRVTITCRASQSISSYLNWYQQKPGKAPKLLIYAASSLQSGVPSRFSGSGSGTDFTLTISSLQPEDFATYYCQQSLDFPPITFGGGTKVEIK

SEQ ID NO: 36 - protein, 13 aa, synthetic construct
LPSSGSYTAHFDY

SEQ ID NO: 37 - protein, 8 aa, synthetic construct
QQGFSFWT

SEQ ID NO: 38 - protein, 122 aa, synthetic construct
EVQLLESGGGLVQPGGSLRLSCAASGFTFSSYAMSWVRQAPGKGLEWVSAISGSGGSTYYADSVKGRFTISRDNSKNTLYLQMNSLRAEDTAVYYCARLPSSGSYTAHFDYWGQGTLVTVSS

SEQ ID NO: 39 - protein, 106 aa, synthetic construct
DIQMTQSPSSVSASVGDRVTITCRASQGISSWLAWYQQKPGKAPKLLIYAASSLQSGVPSRFSGSGSGTDFTLTISSLQPEDFATYYCQQGFSFWTFGGGTKVEIK

SEQ ID NO: 40 - protein, 17 aa, synthetic construct
EGSSSGYSRHGYDYFDY

SEQ ID NO: 41 - protein, 9 aa, synthetic construct
QQYRSYPIT

SEQ ID NO: 42 - protein, 126 aa, synthetic construct
EVQLVESGGGLVQPGRSLRLSCAASGFTFDDYAMHWVRQAPGKGLEWVSGISWNSGSIGYADSVKGRFTISRDNAKNSLYLQMNSLRAEDTAVYYCAREGSSSGYSRHGYDYFDYWGQGTLVTVSS

SEQ ID NO: 43 - protein, 107 aa, synthetic construct
DIQMTQSPSTLSASVGDRVTITCRASQSISSWLAWYQQKPGKAPKLLIYDASSLESGVPSRFSGSGSGTEFTLTISSLQPDDFATYYCQQYRSYPITFGGGTKVEIK

SEQ ID NO: 44 - protein, 10 aa, synthetic construct
GFTFSNFNMK

SEQ ID NO: 45 - protein, 10 aa, synthetic construct
SIISSGGTTG

SEQ ID NO: 46 - protein, 8 aa, synthetic construct
RRRDSEDY

SEQ ID NO: 47 - protein, 117 aa, synthetic construct
QLQLVESGGGLVQPGGSLRLSCAASGFTFSNFNMKWYRQVSGKERELVASIISSGGTTGYADSVKGRFTISRDNAKNTVYLQMNSLKTEDTAVYYCNARRRDSEDYWGQGTQVTVSS

SEQ ID NO: 48 - protein, 10 aa, synthetic construct
GSFFRSIAMA

SEQ ID NO: 49 - protein, 9 aa, synthetic construct
TITSDGDTN

SEQ ID NO: 50 - protein, 6 aa, synthetic construct
PGSIGY

SEQ ID NO: 51 - protein, 114 aa, synthetic construct
QVQLVESGGGLVQPGGSLRLSCAASGSFFRSIAMAWYRQAPGKQRVLVGTITSDGDTNYADSVKGRFTISRDNAKNTMYLQMNSLKPEDTAVYSCNVPGSIGYWSQGTQVTVSS

SEQ ID NO: 52 - protein, 10 aa, synthetic construct
GRTLSSYAMG

SEQ ID NO: 53 - protein, 7 aa, synthetic construct
SIGRSTY

SEQ ID NO: 54 - protein, 14 aa, synthetic construct
PIVAGFGTVVSGEY

SEQ ID NO: 55 - protein, 120 aa, synthetic construct
QVQLVESGGGLVQAGGSLRLSCAASGRTLSSYAMGWFRQAPGKEREFVASIGRSTYYADPVKGRFTISRDNAKNTVYLQMNSLKSEDTAVYYCNAPIVAGFGTVVSGEYWGQGTQVTVSS

SEQ ID NO: 56 - protein, 10 aa, synthetic construct
GSIGNIYDLG

SEQ ID NO: 57 - protein, 9 aa, synthetic construct
SITSGGRTI

SEQ ID NO: 58 - protein, 6 aa, synthetic construct
GHELGY

SEQ ID NO: 59 - protein, 114 aa, synthetic construct
QVQLVESGGGLVQPGESLTLSCTVSGSIGNIYDLGWYRQASGKQRELVASITSGGRTIYADSVEGRFTISRNNAKNTVVLQMNSLEPEDMAVYYCNLGHELGYWGQGTQVTVSS

SEQ ID NO: 60 - protein, 10 aa, synthetic construct
GFTFSTYAMA

SEQ ID NO: 61 - protein, 10 aa, synthetic construct
SIDTSGDNTH

SEQ ID NO: 62 - protein, 10 aa, synthetic construct
PNTGWGTRRY

SEQ ID NO: 63 - protein, 119 aa, synthetic construct
QLQLVESGGGLVQPGGSLRLSCVASGFTFSTYAMAWYRQRPGKERELVASIDTSGDNTHYVGAVKGRFTISRDNAKNTVYLQMNGLKPEDTAVYFCNAPNTGWGTRRYWGQGTQVTVSS

SEQ ID NO: 64 - protein, 10 aa, synthetic construct
GFAFSTYAMA

SEQ ID NO: 65 - protein, 10 aa, synthetic construct
SIDSSGDNTH

SEQ ID NO: 66 - protein, 119 aa, synthetic construct
QLQLVESGGGLVQPGGSLRLSCVASGFAFSTYAMAWYRQRPGKERELVGSIDSSGDNTHYVDAVKGRFTISRDNAKNTVYLQMNVLKPEDTAVYYCNSPNTGWGTRRYWGQGTQVTVSS

SEQ ID NO: 67 - protein, 10 aa, synthetic construct
GFTFSSYAMA

SEQ ID NO: 68 - protein, 10 aa, synthetic construct
SIDSSGYNTH

SEQ ID NO: 69 - protein, 10 aa, synthetic construct
PNTGWGSRRY

SEQ ID NO: 70 - protein, 119 aa, synthetic construct
QLQLVESGGGLVQPGGSLRLSCAASGFTFSSYAMAWYRQRSGKERELVASIDSSGYNTHYTDAGKGRFTISRDNAKNTVYLQMNNLKPEDTAVYYCNAPNTGWGSRRYWGQGTQVTVSS

SEQ ID NO: 71 - protein, 10 aa, synthetic construct
GNIGHIYDLG

SEQ ID NO: 72 - protein, 9 aa, synthetic construct
SITDNGRTI

SEQ ID NO: 73 - protein, 6 aa, synthetic construct
GHWLGY

SEQ ID NO: 74 - protein, 114 aa, synthetic construct
QVQLVESGGGLVQPGESLRLSCSVSGNIGHIYDLGWYRQASGKQRELVASITDNGRTIYGDSVKGRFTISRNNVKNTVNLQMNSLTPEDTAVYYCNLGHWLGYWGQGTQVTVSS

SEQ ID NO: 75 - protein, 120 aa, synthetic construct
QVQLLESGGGLVQAGGSLRLSCAASGRTLSSYAMGWFRQAPGKGLEFVASIGRSTYYADPVKGRFTISRDNSKNTVYLQMNSLRAEDTAVYYCNAPIVAGFGTVVSGEYWGQGTLVTVSS

SEQ ID NO: 76 - protein, 120 aa, synthetic construct
QVQLLESGGGLVQPGGSLRLSCAASGRTLSSYAMGWFRQAPGKGLEFVASIGRSTYYADPVKGRFTISRDNSKNTVYLQMNSLRAEDTAVYYCNAPIVAGFGTVVSGEYWGQGTLVTVSS

SEQ ID NO: 77 - protein, 120 aa, synthetic construct
EVQLLESGGGLVQPGGSLRLSCAASGRTLSSYAMGWFRQAPGKGLEFVASIGRSTYYADPVKGRFTISRDNSKNTVYLQMNSLRAEDTAVYYCNAPIVAGFGTVVSGEYWGQGTLVTVSS

SEQ ID NO: 78 - protein, 120 aa, synthetic construct
QVQLLESGGGLVQPGGSLRLSCAASGRTLSSYAMGWFRQAPGKGLEFVASIGRSTYYADSVKGRFTISRDNSKNTVYLQMNSLRAEDTAVYYCNAPIVAGFGTVVSGEYWGQGTLVTVSS

SEQ ID NO: 79 - protein, 120 aa, synthetic construct
QVQLLESGGGLVQPGGSLRLSCAASGRTLSSYAMGWFRQAPGKGLEFVASIGRSTYYADPVKGRFTISRDNSKNTVYLQMNSLRAEDTAVYYCAAPIVAGFGTVVSGEYWGQGTLVTVSS

SEQ ID NO: 80 - protein, 330 aa, synthetic construct
ASTKGPSVFPLAPSSKSTSGGTAALGCLVKDYFPEPVTVSWNSGALTSGVHTFPAVLQSSGLYSLSSVVTVPSSSLGTQTYICNVNHKPSNTKVDKKVEPKSCDKTHTCPPCPAPELLGGPSVFLFPPKPKDTLMISRTPEVTCVVVDVSHEDPEVKFNWYVDGVEVHNAKTKPREEQYNSTYRVVSVLTVLHQDWLNGKEYKCKVSNKALPAPIEKTISKAKGQPREPQVYTLPPSREEMTKNQVSLTCLVKGFYPSDIAVEWESNGQPENNYKTTPPVLDSDGSFFLYSKLTVDKSRWQQGNVFSCSVMHEALHNHYTQKSLSLSPGK

SEQ ID NO: 81 - protein, 330 aa, synthetic construct
ASTKGPSVFPLAPSSKSTSGGTAALGCLVKDYFPEPVTVSWNSGALTSGVHTFPAVLQSSGLYSLSSVVTVPSSSLGTQTYICNVNHKPSNTKVDKKVEPKSCDKTHTCPPCPAPEAAGGPSVFLFPPKPKDTLMISRTPEVTCVVVDVSHEDPEVKFNWYVDGVEVHNAKTKPREEQYNSTYRVVSVLTVLHQDWLNGKEYKCKVSNKALPAPIEKTISKAKGQPREPQVYTLPPSREEMTKNQVSLTCLVKGFYPSDIAVEWESNGQPENNYKTTPPVLDSDGSFFLYSKLTVDKSRWQQGNVFSCSVMHEALHNHYTQKSLSLSPGK

SEQ ID NO: 82 - protein, 107 aa, synthetic construct [sequence omitted]

SEQ ID NO: 83 - protein, 449 aa, synthetic construct
EVQLVESGGGLVQPGRSLRLSCAASGFTFDDYAMHWVRQAPGKGLEWVSGISWNSGSIGYADSVKGRFTISRDNAKNSLYLQMNSLRAEDTAVYYCARDSGAYVSFDYWGQGTLVTVSSASTKGPSVFPLAPSSKSTSGGTAALGCLVKDYFPEPVTVSWNSGALTSGVHTFPAVLQSSGLYSLSSVVTVPSSSLGTQTYICNVNHKPSNTKVDKKVEPKSCDKTHTCPPCPAPEAAGGPSVFLFPPKPKDTLMISRTPEVTCVVVDVSHEDPEVKFNWYVDGVEVHNAKTKPREEQYNSTYRVVSVLTVLHQDWLNGKEYKCKVSNKALPAPIEKTISKAKGQPREPQVYTLPPSREEMTKNQVSLTCLVKGFYPSDIAVEWESNGQPENNYKTTPPVLDSDGSFFLYSKLTVDKSRWQQGNVFSCSVMHEALHNHYTQKSLSLSPGK

SEQ ID NO: 84 - protein, 215 aa, synthetic construct
DIQMTQSPSSLSASVGDRVTITCRASQSISSYLNWYQQKPGKAPKLLIYAASSLQSGVPSRFSGSGSGTDFTLTISSLQPEDFATYYCQESYSYPPFTFGGGTKVEIKRTVAAPSVFIFPPSDEQLKSGTASVVCLLNNFYPREAKVQWKVDNALQSGNSQESVTEQDSKDSTYSLSSTLTLSKADYEKHKVYACEVTHQGLSSPVTKSFNRGEC

SEQ ID NO: 85 - protein, 449 aa, synthetic construct
EVQLLESGGGLVQPGGSLRLSCAASGFTFSSYAMSWVRQAPGKGLEWVSAISGSGGSTYYADSVKGRFTISRDNSKNTLYLQMNSLRAEDTAVYYCARLEWLYGAFDIWGQGTLVTVSSASTKGPSVFPLAPSSKSTSGGTAALGCLVKDYFPEPVTVSWNSGALTSGVHTFPAVLQSSGLYSLSSVVTVPSSSLGTQTYICNVNHKPSNTKVDKKVEPKSCDKTHTCPPCPAPEAAGGPSVFLFPPKPKDTLMISRTPEVTCVVVDVSHEDPEVKFNWYVDGVEVHNAKTKPREEQYNSTYRVVSVLTVLHQDWLNGKEYKCKVSNKALPAPIEKTISKAKGQPREPQVYTLPPSREEMTKNQVSLTCLVKGFYPSDIAVEWESNGQPENNYKTTPPVLDSDGSFFLYSKLTVDKSRWQQGNVFSCSVMHEALHNHYTQKSLSLSPGK

SEQ ID NO: 86 - protein, 215 aa, synthetic construct
DIQMTQSPSSVSASVGDRVTITCRASQGISSWLAWYQQKPGKAPKLLIYAASSLQSGVPSRFSGSGSGTDFTLTISSLQPEDFATYYCQQADSFPPLTFGGGTKVEIKRTVAAPSVFIFPPSDEQLKSGTASVVCLLNNFYPREAKVQWKVDNALQSGNSQESVTEQDSKDSTYSLSSTLTLSKADYEKHKVYACEVTHQGLSSPVTKSFNRGEC

SEQ ID NO: 87 - protein, 449 aa, synthetic construct
EVQLVESGGGLVQPGRSLRLSCAASGFTFDDYAMHWVRQAPGKGLEWVSGISWNSGSIGYADSVKGRFTISRDNAKNSLYLQMNSLRAEDTAVYYCARSYEDTAHFDYWGQGTLVTVSSASTKGPSVFPLAPSSKSTSGGTAALGCLVKDYFPEPVTVSWNSGALTSGVHTFPAVLQSSGLYSLSSVVTVPSSSLGTQTYICNVNHKPSNTKVDKKVEPKSCDKTHTCPPCPAPEAAGGPSVFLFPPKPKDTLMISRTPEVTCVVVDVSHEDPEVKFNWYVDGVEVHNAKTKPREEQYNSTYRVVSVLTVLHQDWLNGKEYKCKVSNKALPAPIEKTISKAKGQPREPQVYTLPPSREEMTKNQVSLTCLVKGFYPSDIAVEWESNGQPENNYKTTPPVLDSDGSFFLYSKLTVDKSRWQQGNVFSCSVMHEALHNHYTQKSLSLSPGK

SEQ ID NO: 88 - protein, 214 aa, synthetic construct
DIQMTQSPSTLSASVGDRVTITCRASQSISSWLAWYQQKPGKAPKLLIYDASSLESGVPSRFSGSGSGTEFTLTISSLQPDDFATYYCQQYNSFPPTFGGGTKVEIKRTVAAPSVFIFPPSDEQLKSGTASVVCLLNNFYPREAKVQWKVDNALQSGNSQESVTEQDSKDSTYSLSSTLTLSKADYEKHKVYACEVTHQGLSSPVTKSFNRGEC

SEQ ID NO: 89 - protein, 450 aa, synthetic construct
EVQLVESGGGLVQPGRSLRLSCAASGFTFDDYAMHWVRQAPGKGLEWVSGISWNSGSIGYADSVKGRFTISRDNAKNSLYLQMNSLRAEDTAVYYCAKGQVAPLDHFDYWGQGTLVTVSSASTKGPSVFPLAPSSKSTSGGTAALGCLVKDYFPEPVTVSWNSGALTSGVHTFPAVLQSSGLYSLSSVVTVPSSSLGTQTYICNVNHKPSNTKVDKKVEPKSCDKTHTCPPCPAPEAAGGPSVFLFPPKPKDTLMISRTPEVTCVVVDVSHEDPEVKFNWYVDGVEVHNAKTKPREEQYNSTYRVVSVLTVLHQDWLNGKEYKCKVSNKALPAPIEKTISKAKGQPREPQVYTLPPSREEMTKNQVSLTCLVKGFYPSDIAVEWESNGQPENNYKTTPPVLDSDGSFFLYSKLTVDKSRWQQGNVFSCSVMHEALHNHYTQKSLSLSPGK

SEQ ID NO: 90 - protein, 214 aa, synthetic construct
DIQMTQSPSTLSASVGDRVTITCRASQSISSWLAWYQQKPGKAPKLLIYDASSLESGVPSRFSGSGSGTEFTLTISSLQPDDFATYYCEQYNSYPLTFGGGTKVEIKRTVAAPSVFIFPPSDEQLKSGTASVVCLLNNFYPREAKVQWKVDNALQSGNSQESVTEQDSKDSTYSLSSTLTLSKADYEKHKVYACEVTHQGLSSPVTKSFNRGEC

SEQ ID NO: 91 - protein, 450 aa, synthetic construct
QVQLVESGGGVVQPGRSLRLSCAASGFTFSSYAMHWVRQAPGKGLEWVAVISYDGSNKYYADSVKGRFTISRDNSKNTLYLQMNSLRAEDTAVYYCARGQVAILDYFDYWGQGTLVTVSSASTKGPSVFPLAPSSKSTSGGTAALGCLVKDYFPEPVTVSWNSGALTSGVHTFPAVLQSSGLYSLSSVVTVPSSSLGTQTYICNVNHKPSNTKVDKKVEPKSCDKTHTCPPCPAPEAAGGPSVFLFPPKPKDTLMISRTPEVTCVVVDVSHEDPEVKFNWYVDGVEVHNAKTKPREEQYNSTYRVVSVLTVLHQDWLNGKEYKCKVSNKALPAPIEKTISKAKGQPREPQVYTLPPSREEMTKNQVSLTCLVKGFYPSDIAVEWESNGQPENNYKTTPPVLDSDGSFFLYSKLTVDKSRWQQGNVFSCSVMHEALHNHYTQKSLSLSPGK

SEQ ID NO: 92 - protein, 214 aa, synthetic construct
DIQMTQSPSTLSASVGDRVTITCRASQSISSWLAWYQQKPGKAPKLLIYDASSLESGVPSRFSGSGSGTEFTLTISSLQPDDFATYYCQQYNSYPPTFGGGTKVEIKRTVAAPSVFIFPPSDEQLKSGTASVVCLLNNFYPREAKVQWKVDNALQSGNSQESVTEQDSKDSTYSLSSTLTLSKADYEKHKVYACEVTHQGLSSPVTKSFNRGEC

SEQ ID NO: 93 - protein, 450 aa, synthetic construct
EVQLLESGGGLVQPGGSLRLSCAASGFTFSSYAMSWVRQAPGKGLEWVSAISGSGGSTYYADSVKGRFTISRDNSKNTLYLQMNSLRAEDTAVYYCARLGDGVTYAFDIWGQGTLVTVSSASTKGPSVFPLAPSSKSTSGGTAALGCLVKDYFPEPVTVSWNSGALTSGVHTFPAVLQSSGLYSLSSVVTVPSSSLGTQTYICNVNHKPSNTKVDKKVEPKSCDKTHTCPPCPAPEAAGGPSVFLFPPKPKDTLMISRTPEVTCVVVDVSHEDPEVKFNWYVDGVEVHNAKTKPREEQYNSTYRVVSVLTVLHQDWLNGKEYKCKVSNKALPAPIEKTISKAKGQPREPQVYTLPPSREEMTKNQVSLTCLVKGFYPSDIAVEWESNGQPENNYKTTPPVLDSDGSFFLYSKLTVDKSRWQQGNVFSCSVMHEALHNHYTQKSLSLSPGK

SEQ ID NO: 94 - protein, 215 aa, synthetic construct
DIQMTQSPSSLSASVGDRVTITCRASQSISSYLNWYQQKPGKAPKLLIYAASSLQSGVPSRFSGSGSGTDFTLTISSLQPEDFATYYCQQSLDFPPITFGGGTKVEIKRTVAAPSVFIFPPSDEQLKSGTASVVCLLNNFYPREAKVQWKVDNALQSGNSQESVTEQDSKDSTYSLSSTLTLSKADYEKHKVYACEVTHQGLSSPVTKSFNRGEC

SEQ ID NO: 95 - protein, 452 aa, synthetic construct
EVQLLESGGGLVQPGGSLRLSCAASGFTFSSYAMSWVRQAPGKGLEWVSAISGSGGSTYYADSVKGRFTISRDNSKNTLYLQMNSLRAEDTAVYYCARLPSSGSYTAHFDYWGQGTLVTVSSASTKGPSVFPLAPSSKSTSGGTAALGCLVKDYFPEPVTVSWNSGALTSGVHTFPAVLQSSGLYSLSSVVTVPSSSLGTQTYICNVNHKPSNTKVDKKVEPKSCDKTHTCPPCPAPEAAGGPSVFLFPPKPKDTLMISRTPEVTCVVVDVSHEDPEVKFNWYVDGVEVHNAKTKPREEQYNSTYRVVSVLTVLHQDWLNGKEYKCKVSNKALPAPIEKTISKAKGQPREPQVYTLPPSREEMTKNQVSLTCLVKGFYPSDIAVEWESNGQPENNYKTTPPVLDSDGSFFLYSKLTVDKSRWQQGNVFSCSVMHEALHNHYTQKSLSLSPGK

SEQ ID NO: 96 - protein, 213 aa, synthetic construct
DIQMTQSPSSVSASVGDRVTITCRASQGISSWLAWYQQKPGKAPKLLIYAASSLQSGVPSRFSGSGSGTDFTLTISSLQPEDFATYYCQQGFSFWTFGGGTKVEIKRTVAAPSVFIFPPSDEQLKSGTASVVCLLNNFYPREAKVQWKVDNALQSGNSQESVTEQDSKDSTYSLSSTLTLSKADYEKHKVYACEVTHQGLSSPVTKSFNRGEC

SEQ ID NO: 97 - protein, 456 aa, synthetic construct
EVQLVESGGGLVQPGRSLRLSCAASGFTFDDYAMHWVRQAPGKGLEWVSGISWNSGSIGYADSVKGRFTISRDNAKNSLYLQMNSLRAEDTAVYYCAREGSSSGYSRHGYDYFDYWGQGTLVTVSSASTKGPSVFPLAPSSKSTSGGTAALGCLVKDYFPEPVTVSWNSGALTSGVHTFPAVLQSSGLYSLSSVVTVPSSSLGTQTYICNVNHKPSNTKVDKKVEPKSCDKTHTCPPCPAPEAAGGPSVFLFPPKPKDTLMISRTPEVTCVVVDVSHEDPEVKFNWYVDGVEVHNAKTKPREEQYNSTYRVVSVLTVLHQDWLNGKEYKCKVSNKALPAPIEKTISKAKGQPREPQVYTLPPSREEMTKNQVSLTCLVKGFYPSDIAVEWESNGQPENNYKTTPPVLDSDGSFFLYSKLTVDKSRWQQGNVFSCSVMHEALHNHYTQKSLSLSPGK

SEQ ID NO: 98 - protein, 214 aa, synthetic construct
DIQMTQSPSTLSASVGDRVTITCRASQSISSWLAWYQQKPGKAPKLLIYDASSLESGVPSRFSGSGSGTEFTLTISSLQPDDFATYYCQQYRSYPITFGGGTKVEIKRTVAAPSVFIFPPSDEQLKSGTASVVCLLNNFYPREAKVQWKVDNALQSGNSQESVTEQDSKDSTYSLSSTLTLSKADYEKHKVYACEVTHQGLSSPVTKSFNRGEC

SEQ ID NO: 99 - protein, 232 aa, synthetic construct
EPKSCDKTHTCPPCPAPELLGGPSVFLFPPKPKDTLMISRTPEVTCVVVDVSHEDPEVKFNWYVDGVEVHNAKTKPREEQYNSTYRVVSVLTVLHQDWLNGKEYKCKVSNKALPAPIEKTISKAKGQPREPQVYTLPPSREEMTKNQVSLTCLVKGFYPSDIAVEWESNGQPENNYKTTPPVLDSDGSFFLYSKLTVDKSRWQQGNVFSCSVMHEALHNHYTQKSLSLSPGK

SEQ ID NO: 100 - protein, 232 aa, synthetic construct
EPKSADKTHTCPPCPAPEAAGGPSVFLFPPKPKDTLMISRTPEVTCVVVDVSHEDPEVKFNWYVDGVEVHNAKTKPREEQYNSTYRVVSVLTVLHQDWLNGKEYKCKVSNKALPAPIEKTISKAKGQPREPQVYTLPPSREEMTKNQVSLTCLVKGFYPSDIAVEWESNGQPENNYKTTPPVLDSDGSFFLYSKLTVDKSRWQQGNVFSCSVMHEALHNHYTQKSLSLSPGK

SEQ ID NO: 101 - protein, 349 aa, synthetic construct
QLQLVESGGGLVQPGGSLRLSCAASGFTFSNFNMKWYRQVSGKERELVASIISSGGTTGYADSVKGRFTISRDNAKNTVYLQMNSLKTEDTAVYYCNARRRDSEDYWGQGTQVTVSSEPKSADKTHTCPPCPAPEAAGGPSVFLFPPKPKDTLMISRTPEVTCVVVDVSHEDPEVKFNWYVDGVEVHNAKTKPREEQYNSTYRVVSVLTVLHQDWLNGKEYKCKVSNKALPAPIEKTISKAKGQPREPQVYTLPPSREEMTKNQVSLTCLVKGFYPSDIAVEWESNGQPENNYKTTPPVLDSDGSFFLYSKLTVDKSRWQQGNVFSCSVMHEALHNHYTQKSLSLSPGK

SEQ ID NO: 102 - protein, 346 aa, synthetic construct
QVQLVESGGGLVQPGGSLRLSCAASGSFFRSIAMAWYRQAPGKQRVLVGTITSDGDTNYADSVKGRFTISRDNAKNTMYLQMNSLKPEDTAVYSCNVPGSIGYWSQGTQVTVSSEPKSADKTHTCPPCPAPEAAGGPSVFLFPPKPKDTLMISRTPEVTCVVVDVSHEDPEVKFNWYVDGVEVHNAKTKPREEQYNSTYRVVSVLTVLHQDWLNGKEYKCKVSNKALPAPIEKTISKAKGQPREPQVYTLPPSREEMTKNQVSLTCLVKGFYPSDIAVEWESNGQPENNYKTTPPVLDSDGSFFLYSKLTVDKSRWQQGNVFSCSVMHEALHNHYTQKSLSLSPGK

SEQ ID NO: 103 - protein, 352 aa, synthetic construct
QVQLVESGGGLVQAGGSLRLSCAASGRTLSSYAMGWFRQAPGKEREFVASIGRSTYYADPVKGRFTISRDNAKNTVYLQMNSLKSEDTAVYYCNAPIVAGFGTVVSGEYWGQGTQVTVSSEPKSADKTHTCPPCPAPEAAGGPSVFLFPPKPKDTLMISRTPEVTCVVVDVSHEDPEVKFNWYVDGVEVHNAKTKPREEQYNSTYRVVSVLTVLHQDWLNGKEYKCKVSNKALPAPIEKTISKAKGQPREPQVYTLPPSREEMTKNQVSLTCLVKGFYPSDIAVEWESNGQPENNYKTTPPVLDSDGSFFLYSKLTVDKSRWQQGNVFSCSVMHEALHNHYTQKSLSLSPGK

SEQ ID NO: 104 - protein, 346 aa, synthetic construct
QVQLVESGGGLVQPGESLTLSCTVSGSIGNIYDLGWYRQASGKQRELVASITSGGRTIYADSVEGRFTISRNNAKNTVVLQMNSLEPEDMAVYYCNLGHELGYWGQGTQVTVSSEPKSADKTHTCPPCPAPEAAGGPSVFLFPPKPKDTLMISRTPEVTCVVVDVSHEDPEVKFNWYVDGVEVHNAKTKPREEQYNSTYRVVSVLTVLHQDWLNGKEYKCKVSNKALPAPIEKTISKAKGQPREPQVYTLPPSREEMTKNQVSLTCLVKGFYPSDIAVEWESNGQPENNYKTTPPVLDSDGSFFLYSKLTVDKSRWQQGNVFSCSVMHEALHNHYTQKSLSLSPGK

SEQ ID NO: 105 - protein, 351 aa, synthetic construct
QLQLVESGGGLVQPGGSLRLSCVASGFTFSTYAMAWYRQRPGKERELVASIDTSGDNTHYVGAVKGRFTISRDNAKNTVYLQMNGLKPEDTAVYFCNAPNTGWGTRRYWGQGTQVTVSSEPKSADKTHTCPPCPAPEAAGGPSVFLFPPKPKDTLMISRTPEVTCVVVDVSHEDPEVKFNWYVDGVEVHNAKTKPREEQYNSTYRVVSVLTVLHQDWLNGKEYKCKVSNKALPAPIEKTISKAKGQPREPQVYTLPPSREEMTKNQVSLTCLVKGFYPSDIAVEWESNGQPENNYKTTPPVLDSDGSFFLYSKLTVDKSRWQQGNVFSCSVMHEALHNHYTQKSLSLSPGK

SEQ ID NO: 106 - protein, 351 aa, synthetic construct
QLQLVESGGGLVQPGGSLRLSCVASGFAFSTYAMAWYRQRPGKERELVGSIDSSGDNTHYVDAVKGRFTISRDNAKNTVYLQMNVLKPEDTAVYYCNSPNTGWGTRRYWGQGTQVTVSSEPKSADKTHTCPPCPAPEAAGGPSVFLFPPKPKDTLMISRTPEVTCVVVDVSHEDPEVKFNWYVDGVEVHNAKTKPREEQYNSTYRVVSVLTVLHQDWLNGKEYKCKVSNKALPAPIEKTISKAKGQPREPQVYTLPPSREEMTKNQVSLTCLVKGFYPSDIAVEWESNGQPENNYKTTPPVLDSDGSFFLYSKLTVDKSRWQQGNVFSCSVMHEALHNHYTQKSLSLSPGK

SEQ ID NO: 107 - protein, 351 aa, synthetic construct
QLQLVESGGGLVQPGGSLRLSCAASGFTFSSYAMAWYRQRSGKERELVASIDSSGYNTHYTDAGKGRFTISRDNAKNTVYLQMNNLKPEDTAVYYCNAPNTGWGSRRYWGQGTQVTVSSEPKSADKTHTCPPCPAPEAAGGPSVFLFPPKPKDTLMISRTPEVTCVVVDVSHEDPEVKFNWYVDGVEVHNAKTKPREEQYNSTYRVVSVLTVLHQDWLNGKEYKCKVSNKALPAPIEKTISKAKGQPREPQVYTLPPSREEMTKNQVSLTCLVKGFYPSDIAVEWESNGQPENNYKTTPPVLDSDGSFFLYSKLTVDKSRWQQGNVFSCSVMHEALHNHYTQKSLSLSPGK

SEQ ID NO: 108 - protein, 346 aa, synthetic construct
QVQLVESGGGLVQPGESLRLSCSVSGNIGHIYDLGWYRQASGKQRELVASITDNGRTIYGDSVKGRFTISRNNVKNTVNLQMNSLTPEDTAVYYCNLGHWLGYWGQGTQVTVSSEPKSADKTHTCPPCPAPEAAGGPSVFLFPPKPKDTLMISRTPEVTCVVVDVSHEDPEVKFNWYVDGVEVHNAKTKPREEQYNSTYRVVSVLTVLHQDWLNGKEYKCKVSNKALPAPIEKTISKAKGQPREPQVYTLPPSREEMTKNQVSLTCLVKGFYPSDIAVEWESNGQPENNYKTTPPVLDSDGSFFLYSKLTVDKSRWQQGNVFSCSVMHEALHNHYTQKSLSLSPGK

SEQ ID NO: 109 - protein, 352 aa, synthetic construct
QVQLLESGGGLVQAGGSLRLSCAASGRTLSSYAMGWFRQAPGKGLEFVASIGRSTYYADPVKGRFTISRDNSKNTVYLQMNSLRAEDTAVYYCNAPIVAGFGTVVSGEYWGQGTLVTVSSEPKSADKTHTCPPCPAPEAAGGPSVFLFPPKPKDTLMISRTPEVTCVVVDVSHEDPEVKFNWYVDGVEVHNAKTKPREEQYNSTYRVVSVLTVLHQDWLNGKEYKCKVSNKALPAPIEKTISKAKGQPREPQVYTLPPSREEMTKNQVSLTCLVKGFYPSDIAVEWESNGQPENNYKTTPPVLDSDGSFFLYSKLTVDKSRWQQGNVFSCSVMHEALHNHYTQKSLSLSPGK

SEQ ID NO: 110 - protein, 352 aa, synthetic construct
QVQLLESGGGLVQPGGSLRLSCAASGRTLSSYAMGWFRQAPGKGLEFVASIGRSTYYADPVKGRFTISRDNSKNTVYLQMNSLRAEDTAVYYCNAPIVAGFGTVVSGEYWGQGTLVTVSSEPKSADKTHTCPPCPAPEAAGGPSVFLFPPKPKDTLMISRTPEVTCVVVDVSHEDPEVKFNWYVDGVEVHNAKTKPREEQYNSTYRVVSVLTVLHQDWLNGKEYKCKVSNKALPAPIEKTISKAKGQPREPQVYTLPPSREEMTKNQVSLTCLVKGFYPSDIAVEWESNGQPENNYKTTPPVLDSDGSFFLYSKLTVDKSRWQQGNVFSCSVMHEALHNHYTQKSLSLSPGK

SEQ ID NO: 111 - protein, 352 aa, synthetic construct
EVQLLESGGGLVQPGGSLRLSCAASGRTLSSYAMGWFRQAPGKGLEFVASIGRSTYYADPVKGRFTISRDNSKNTVYLQMNSLRAEDTAVYYCNAPIVAGFGTVVSGEYWGQGTLVTVSSEPKSADKTHTCPPCPAPEAAGGPSVFLFPPKPKDTLMISRTPEVTCVVVDVSHEDPEVKFNWYVDGVEVHNAKTKPREEQYNSTYRVVSVLTVLHQDWLNGKEYKCKVSNKALPAPIEKTISKAKGQPREPQVYTLPPSREEMTKNQVSLTCLVKGFYPSDIAVEWESNGQPENNYKTTPPVLDSDGSFFLYSKLTVDKSRWQQGNVFSCSVMHEALHNHYTQKSLSLSPGK

SEQ ID NO: 112 - protein, 352 aa, synthetic construct
QVQLLESGGGLVQPGGSLRLSCAASGRTLSSYAMGWFRQAPGKGLEFVASIGRSTYYADSVKGRFTISRDNSKNTVYLQMNSLRAEDTAVYYCNAPIVAGFGTVVSGEYWGQGTLVTVSSEPKSADKTHTCPPCPAPEAAGGPSVFLFPPKPKDTLMISRTPEVTCVVVDVSHEDPEVKFNWYVDGVEVHNAKTKPREEQYNSTYRVVSVLTVLHQDWLNGKEYKCKVSNKALPAPIEKTISKAKGQPREPQVYTLPPSREEMTKNQVSLTCLVKGFYPSDIAVEWESNGQPENNYKTTPPVLDSDGSFFLYSKLTVDKSRWQQGNVFSCSVMHEALHNHYTQKSLSLSPGK

SEQ ID NO: 113 - protein, 352 aa, synthetic construct
QVQLLESGGGLVQPGGSLRLSCAASGRTLSSYAMGWFRQAPGKGLEFVASIGRSTYYADPVKGRFTISRDNSKNTVYLQMNSLRAEDTAVYYCAAPIVAGFGTVVSGEYWGQGTLVTVSSEPKSADKTHTCPPCPAPEAAGGPSVFLFPPKPKDTLMISRTPEVTCVVVDVSHEDPEVKFNWYVDGVEVHNAKTKPREEQYNSTYRVVSVLTVLHQDWLNGKEYKCKVSNKALPAPIEKTISKAKGQPREPQVYTLPPSREEMTKNQVSLTCLVKGFYPSDIAVEWESNGQPENNYKTTPPVLDSDGSFFLYSKLTVDKSRWQQGNVFSCSVMHEALHNHYTQKSLSLSPGK

SEQ ID NO: 114 - protein, 329 aa, synthetic construct
ASTKGPSVFPLAPSSKSTSGGTAALGCLVKDYFPEPVTVSWNSGALTSGVHTFPAVLQSSGLYSLSSVVTVPSSSLGTQTYICNVNHKPSNTKVDKKVEPKSCDKTHTCPPCPAPEAAGGPSVFLFPPKPKDTLYITREPEVTCVVVDVSHEDPEVKFNWYVDGVEVHNAKTKPREEQYNSTYRVVSVLTVLHQDWLNGKEYKCKVSNKALPAPIEKTISKAKGQPREPQVYTLPPSREEMTKNQVSLTCLVKGFYPSDIAVEWESNGQPENNYKTTPPVLDSDGSFFLYSKLTVDKSRWQQGNVFSCSVMHEALHNHYTQKSLSLSPG

SEQ ID NO: 115 - protein, 585 aa, synthetic construct
QVQLVESGGGVVQPGRSLRLSCAASGFTFSSYAMHWVRQAPGKGLEWVAVISYDGSNKYYADSVKGRFTISRDNSKNTLYLQMNSLRAEDTAVYYCARGQVAILDYFDYWGQGTLVTVSSASTKGPSVFPLAPSSKSTSGGTAALGCLVKDYFPEPVTVSWNSGALTSGVHTFPAVLQSSGLYSLSSVVTVPSSSLGTQTYICNVNHKPSNTKVDKKVEPKSCDKTHTCPPCPAPEAAGGPSVFLFPPKPKDTLYITREPEVTCVVVDVSHEDPEVKFNWYVDGVEVHNAKTKPREEQYNSTYRVVSVLTVLHQDWLNGKEYKCKVSNKALPAPIEKTISKAKGQPREPQVYTLPPSREEMTKNQVSLTCLVKGFYPSDIAVEWESNGQPENNYKTTPPVLDSDGSFFLYSKLTVDKSRWQQGNVFSCSVMHEALHNHYTQKSLSLSPGGGGGSGGGGSGGGGSEVQLLESGGGLVQPGGSLRLSCAASGRTLSSYAMGWFRQAPGKGLEFVASIGRSTYYADPVKGRFTISRDNSKNTVYLQMNSLRAEDTAVYYCNAPIVAGFGTVVSGEYWGQGTLVTVSSA

SEQ ID NO: 116 - protein, 590 aa, synthetic construct
QVQLVESGGGVVQPGRSLRLSCAASGFTFSSYAMHWVRQAPGKGLEWVAVISYDGSNKYYADSVKGRFTISRDNSKNTLYLQMNSLRAEDTAVYYCARGQVAILDYFDYWGQGTLVTVSSASTKGPSVFPLAPSSKSTSGGTAALGCLVKDYFPEPVTVSWNSGALTSGVHTFPAVLQSSGLYSLSSVVTVPSSSLGTQTYICNVNHKPSNTKVDKKVEPKSCDKTHTCPPCPAPEAAGGPSVFLFPPKPKDTLYITREPEVTCVVVDVSHEDPEVKFNWYVDGVEVHNAKTKPREEQYNSTYRVVSVLTVLHQDWLNGKEYKCKVSNKALPAPIEKTISKAKGQPREPQVYTLPPSREEMTKNQVSLTCLVKGFYPSDIAVEWESNGQPENNYKTTPPVLDSDGSFFLYSKLTVDKSRWQQGNVFSCSVMHEALHNHYTQKSLSLSPGGGGGSGGGGSGGGGSGGGGSEVQLLESGGGLVQPGGSLRLSCAASGRTLSSYAMGWFRQAPGKGLEFVASIGRSTYYADPVKGRFTISRDNSKNTVYLQMNSLRAEDTAVYYCNAPIVAGFGTVVSGEYWGQGTLVTVSSA

SEQ ID NO: 117 - protein, 98 aa, synthetic construct
ASTKGPSVFPLAPSSKSTSGGTAALGCLVKDYFPEPVTVSWNSGALTSGVHTFPAVLQSSGLYSLSSVVTVPSSSLGTQTYICNVNHKPSNTKVDKKV

SEQ ID NO: 118 - protein, 232 aa, synthetic construct
EPKSCDKTHTCPPCPAPEAAGGPSVFLFPPKPKDTLMISRTPEVTCVVVDVSHEDPEVKFNWYVDGVEVHNAKTKPREEQYNSTYRVVSVLTVLHQDWLNGKEYKCKVSNKALPAPIEKTISKAKGQPREPQVYTLPPSREEMTKNQVSLTCLVKGFYPSDIAVEWESNGQPENNYKTTPPVLDSDGSFFLYSKLTVDKSRWQQGNVFSCSVMHEALHNHYTQKSLSLSPGK

SEQ ID NO: 119 - protein, 231 aa, synthetic construct
EPKSCDKTHTCPPCPAPEAAGGPSVFLFPPKPKDTLYITREPEVTCVVVDVSHEDPEVKFNWYVDGVEVHNAKTKPREEQYNSTYRVVSVLTVLHQDWLNGKEYKCKVSNKALPAPIEKTISKAKGQPREPQVYTLPPSREEMTKNQVSLTCLVKGFYPSDIAVEWESNGQPENNYKTTPPVLDSDGSFFLYSKLTVDKSRWQQGNVFSCSVMHEALHNHYTQKSLSLSPG